European Patent Application EP 4 434 341 A1, published September 25, 2024. Title: 一种新的改善血小板质量的方法. Applicant: 上海循曜生物科技有限公司. The sequence listing filed with the application follows.

SEQUENCE LISTING (12 sequences)

SEQ ID NO: 1 - DNA, 23 bp, synthetic construct
  source 1..23: mol_type = other DNA
tgtgttttcttgaaaattacagg

SEQ ID NO: 2 - DNA, 23 bp, synthetic construct
  source 1..23: mol_type = other DNA
gaagacagaagtgttgtgtaagg

SEQ ID NO: 3 - DNA, 76 bp, synthetic construct
  source 1..76: mol_type = other DNA
gtggtttgacctgtgttttcttgaaaattacagacagacagaggtgttgtgtaaggattttgagaacggcattggg

SEQ ID NO: 4 - DNA, 76 bp, synthetic construct
  source 1..76: mol_type = other DNA
gtggtttgacctgtgttttcttgaaaattacagaaggacagaggtgttgtgtaaggattttgagaacggcattggg

SEQ ID NO: 5 - DNA, 23 bp, synthetic construct
  source 1..23: mol_type = other DNA
tgtgttttcttgaaaattacagg

SEQ ID NO: 6 - DNA, 23 bp, synthetic construct
  source 1..23: mol_type = other DNA
gaagacagaagtgttgtgtaagg

SEQ ID NO: 7 - DNA, 76 bp, synthetic construct; identical to SEQ ID NO: 4
  source 1..76: mol_type = other DNA

SEQ ID NO: 8 - DNA, 22 bp, synthetic construct
  source 1..22: mol_type = other DNA
scttctgcggctctatacacag

SEQ ID NO: 9 - DNA, 20 bp, synthetic construct
  source 1..20: mol_type = other DNA
tgcaacaaggcttatcttcc

SEQ ID NO: 10 - DNA, 21 bp, synthetic construct
  source 1..21: mol_type = other DNA
tactgaatatcagtgggaacg

SEQ ID NO: 11 - DNA, 19 bp, synthetic construct
  source 1..19: mol_type = other DNA
ctttcctcggtgcctctgt

SEQ ID NO: 12 - DNA, 19 bp, synthetic construct
  source 1..19: mol_type = other DNA
cttcccaatgccgttctca